European Patent Application EP 4 198 145 A1, published June 21, 2023. Title: LAMP ASSAY DEVICE AND METHOD THAT PROMOTES ISOTHEMAL AMPLIFICATION OF RNA/DNA APPLIED TO PATHOGEN IDENTIFICATION. Applicant: FUNDACAO OSWALDO CRUZ. The sequence listing filed with the application follows.

SEQUENCE LISTING (72 sequences)

SEQ ID NO: 1 - DNA, 20 bp, Artificial Sequence
  External type primer for isothermal mediated amplification by Zika virus loop
gcagagcaatggatgggata

SEQ ID NO: 2 - DNA, 20 bp, Artificial Sequence
  External type primer for isothermal mediated amplification by Zika virus loop
cccatccttgaggtacagct

SEQ ID NO: 3 - DNA, 41 bp, Artificial Sequence
  Internal type primer for isothermal amplification mediated by Zika virus loop
aacctgagggcatgtgcaaaccgcggtcagtggagatgact

SEQ ID NO: 4 - DNA, 41 bp, Artificial Sequence
  Internal type primer for isothermal amplification mediated by Zika virus loop
cacaggagtggaaaccctcgactgaagtggtgggagcagaa

SEQ ID NO: 5 - DNA, 19 bp, Artificial Sequence
  Loop type primer for isothermal amplification mediated by Zika virus loop
tcgattggcttcacaacgc

SEQ ID NO: 6 - DNA, 21 bp, Artificial Sequence
  Loop type primer for isothermal amplification mediated by Zika virus loop
ggagcaattgggaagaagtcc

SEQ ID NO: 7 - DNA, 18 bp, Artificial Sequence
  External type primer for isothermal mediated amplification by Dengue virus loop
gctgtacgcacggtgtag

SEQ ID NO: 8 - DNA, 20 bp, Artificial Sequence
  External type primer for isothermal mediated amplification by Dengue virus loop
cctggaatgatgctgaggag

SEQ ID NO: 9 - DNA, 41 bp, Artificial Sequence
  Internal type primer for isothermal amplification mediated by Dengue virus loop
ggtacagcttccctcagtgctcgtggttagaggagacccct

SEQ ID NO: 10 - DNA, 41 bp, Artificial Sequence
  Internal type primer for isothermal amplification mediated by Dengue virus loop
agaggttagaggagaccccccagcaggatctctggtctctc

SEQ ID NO: 11 - DNA, 17 bp, Artificial Sequence
  Loop type primer for isothermal amplification mediated by Dengue virus loop
ctgctgcgttgtgtcat

SEQ ID NO: 12 - DNA, 17 bp, Artificial Sequence
  Loop type primer for isothermal amplification mediated by Dengue virus loop
cagcatattgacgctgg

SEQ ID NO: 13 - DNA, 18 bp, Artificial Sequence
  External type primer for isothermal mediated amplification by Chikungunya virus loop
cgtcaacgtactcctaac

SEQ ID NO: 14 - DNA, 18 bp, Artificial Sequence
  External type primer for isothermal mediated amplification by Chikungunya virus loop
acgttggctttrttttgg

SEQ ID NO: 15 - DNA, 40 bp, Artificial Sequence
  Internal type primer for isothermal amplification mediated by Chikungunya virus loop
gaagtttcctttcggtgggtttttggaagacactytcygg

SEQ ID NO: 16 - DNA, 39 bp, Artificial Sequence
  Internal type primer for isothermal amplification mediated by Chikungunya virus loop
aaggagtgggaggtggattttttcayttggtgactgcag

SEQ ID NO: 17 - DNA, 18 bp, Artificial Sequence
  Loop type primer for isothermal amplification mediated by Chikungunya virus loop
agcgtctttatccacggg

SEQ ID NO: 18 - DNA, 19 bp, Artificial Sequence
  Loop type primer for isothermal amplification mediated by Chikungunya virus loop
aygcatcrataatggcggg

SEQ ID NO: 19 - DNA, 20 bp, Artificial Sequence
  External type primer for isothermal mediated amplification by yellow fever virus loop
tccacaccttggaggcatta

SEQ ID NO: 20 - DNA, 20 bp, Artificial Sequence
  External type primer for isothermal mediated amplification by yellow fever virus loop
gtccatcacagttgccatca

SEQ ID NO: 21 - DNA, 38 bp, Artificial Sequence
  Internal type primer for isothermal amplification mediated by yellow fever virus loop
ggcctccgattgatctcggcgtgtgagtggccactgac

SEQ ID NO: 22 - DNA, 40 bp, Artificial Sequence
  Internal type primer for isothermal amplification mediated by yellow fever virus loop
ggttcagacgaacggaccttggccctgggcaagcttctct

SEQ ID NO: 23 - DNA, 25 bp, Artificial Sequence
  Loop type primer for isothermal amplification mediated by yellow fever virus loop
cttcaactgatgttccaatcgtatg

SEQ ID NO: 24 - DNA, 22 bp, Artificial Sequence
  Loop type primer for isothermal amplification mediated by yellow fever virus loop
atgcaggtaccactagaagtga

SEQ ID NO: 25 - DNA, 19 bp, Artificial Sequence
  External type primer for isothermal mediated amplification by SARS-Cov-2 N region loop
tggctactaccgaagagct

SEQ ID NO: 26 - DNA, 20 bp, Artificial Sequence
  External type primer for isothermal mediated amplification by SARS-Cov-2 N region loop
tgcagcattgttagcaggat

SEQ ID NO: 27 - DNA, 41 bp, Artificial Sequence
  Internal type primer for isothermal amplification mediated by SARS-Cov-2 N region loop
tctggcccagttcctaggtagtgacgaattcgtggtggtga

SEQ ID NO: 28 - DNA, 40 bp, Artificial Sequence
  Internal type primer for isothermal amplification mediated by SARS-Cov-2 N region loop
agacggcatcatatgggttgcacgggtgccaatgtgatct

SEQ ID NO: 29 - DNA, 25 bp, Artificial Sequence
  Loop type primer for isothermal amplification mediated by SARS-Cov-2 N region loop
tggactgagatctttcattttaccg

SEQ ID NO: 30 - DNA, 21 bp, Artificial Sequence
  Loop type primer for isothermal amplification mediated by SARS-Cov-2 N region loop
actgagggagccttgaataca

SEQ ID NO: 31 - DNA, 18 bp, Artificial Sequence
  External type primer for isothermal mediated amplification by SARS-Cov-2 N region loop
tggaccccaaaatcagcg

SEQ ID NO: 32 - DNA, 19 bp, Artificial Sequence
  External type primer for isothermal mediated amplification by SARS-Cov-2 N region loop
gccttgtcctcgagggaat

SEQ ID NO: 33 - DNA, 41 bp, Artificial Sequence
  Internal type primer for isothermal amplification mediated by SARS-Cov-2 N region loop
ccactgcgttctccattctggtaaatgcaccccgcattacg

SEQ ID NO: 34 - DNA, 41 bp, Artificial Sequence
  Internal type primer for isothermal amplification mediated by SARS-Cov-2 N region loop
cgcgatcaaaacaacgtcggcccttgccatgttgagtgaga

SEQ ID NO: 35 - DNA, 21 bp, Artificial Sequence
  Loop type primer for isothermal amplification mediated by SARS-Cov-2 N region loop
tgaatctgagggtccaccaaa

SEQ ID NO: 36 - DNA, 25 bp, Artificial Sequence
  Loop type primer for isothermal amplification mediated by SARS-Cov-2 N region loop
ggtttacccaataatactgcgtctt

SEQ ID NO: 37 - DNA, 20 bp, Artificial Sequence
  External type primer for isothermal mediated amplification by SARS-Cov-2 E region loop
tgatgagcctgaagaacatg

SEQ ID NO: 38 - DNA, 23 bp, Artificial Sequence
  External type primer for isothermal mediated amplification by SARS-Cov-2 E region loop
cgctattaactattaacgtacct

SEQ ID NO: 39 - DNA, 45 bp, Artificial Sequence
  Internal type primer for isothermal amplification mediated by SARS-Cov-2 E region loop
tcggttcatcataaattggttccatcaaattcacacaatcgacgg

SEQ ID NO: 40 - DNA, 39 bp, Artificial Sequence
  Internal type primer for isothermal amplification mediated by SARS-Cov-2 E region loop
acgactactagcgtgcctttgtctcttccgaaacgaatg

SEQ ID NO: 41 - DNA, 23 bp, Artificial Sequence
  Loop type primer for isothermal amplification mediated by SARS-Cov-2 E region loop
actggattaacaactccggatga

SEQ ID NO: 42 - DNA, 25 bp, Artificial Sequence
  Loop type primer for isothermal amplification mediated by SARS-Cov-2 E region loop
gtaagcacaagctgatgagtacgaa

SEQ ID NO: 43 - DNA, 19 bp, Artificial Sequence
  External type primer for isothermal mediated amplification by SARS-Cov-2 E region loop
ttgtaagcacaagctgatg

SEQ ID NO: 44 - DNA, 23 bp, Artificial Sequence
  External type primer for isothermal mediated amplification by SARS-Cov-2 E region loop
agagtaaacgtaaaaagaaggtt

SEQ ID NO: 45 - DNA, 49 bp, Artificial Sequence
  Internal type primer for isothermal amplification mediated by SARS-Cov-2 E region loop
cgaaagcaagaaaaagaagtacgctagtacgaacttatgtactcattcg

SEQ ID NO: 46 - DNA, 48 bp, Artificial Sequence
  Internal type primer for isothermal amplification mediated by SARS-Cov-2 E region loop
tggtattcttgctagttacactagcaagactcacgttaacaatattgc

SEQ ID NO: 47 - DNA, 21 bp, Artificial Sequence
  Loop type primer for isothermal amplification mediated by SARS-Cov-2 E region loop
acgtacctgtctcttccgaaa

SEQ ID NO: 48 - DNA, 21 bp, Artificial Sequence
  Loop type primer for isothermal amplification mediated by SARS-Cov-2 E region loop
catccttactgcgcttcgatt

SEQ ID NO: 49 - DNA, 24 bp, Artificial Sequence
  External type primer for isothermal mediated amplification by SARS-Cov-2 RdRp region loop
ctgtcaaattacagaataatgagc

SEQ ID NO: 50 - DNA, 20 bp, Artificial Sequence
  External type primer for isothermal mediated amplification by SARS-Cov-2 RdRp region loop
tccatcactcttagggaatc

SEQ ID NO: 51 - DNA, 40 bp, Artificial Sequence
  Internal type primer for isothermal amplification mediated by SARS-Cov-2 RdRp region loop
tgtcatcagtgcaagcagtttgctgttgcactacgacaga

SEQ ID NO: 52 - DNA, 46 bp, Artificial Sequence
  Internal type primer for isothermal amplification mediated by SARS-Cov-2 RdRp region loop
atgcgttagcttactacaacacacccatttcaaatcctgtaaatcg

SEQ ID NO: 53 - DNA, 17 bp, Artificial Sequence
  Loop type primer for isothermal amplification mediated by SARS-Cov-2 RdRp region loop
accggcagcacaagaca

SEQ ID NO: 54 - DNA, 23 bp, Artificial Sequence
  Loop type primer for isothermal amplification mediated by SARS-Cov-2 RdRp region loop
acaaagggaggtaggtttgtact

SEQ ID NO: 55 - DNA, 21 bp, Artificial Sequence
  External type primer for isothermal mediated amplification by SARS-Cov-2 N2 region loop
accaggaactaatcagacaag

SEQ ID NO: 56 - DNA, 25 bp, Artificial Sequence
  External type primer for isothermal mediated amplification by SARS-Cov-2 N2 region loop
gacttgatctttgaaatttggatct

SEQ ID NO: 57 - DNA, 42 bp, Artificial Sequence
  Internal type primer for isothermal amplification mediated by SARS-Cov-2 N2 region loop
ttccgaagaacgctgaagcggaactgattacaaacattggcc

SEQ ID NO: 58 - DNA, 40 bp, Artificial Sequence
  Internal type primer for isothermal amplification mediated by SARS-Cov-2 N2 region loop
cgcattggcatggaagtcacaatttgatggcacctgtgta

SEQ ID NO: 59 - DNA, 21 bp, Artificial Sequence
  Loop type primer for isothermal amplification mediated by SARS-Cov-2 N2 region loop
gggggcaaattgtgcaatttg

SEQ ID NO: 60 - DNA, 20 bp, Artificial Sequence
  Loop type primer for isothermal amplification mediated by SARS-Cov-2 N2 region loop
cttcgggaacgtggttgacc

SEQ ID NO: 61 - DNA, 23 bp, Artificial Sequence
  External type primer for isothermal mediated amplification by SARS-Cov-2 E1 region loop
tgagtacgaacttatgtactcat

SEQ ID NO: 62 - DNA, 22 bp, Artificial Sequence
  External type primer for isothermal mediated amplification by SARS-Cov-2 E1 region loop
ttcagatttttaacacgagagt

SEQ ID NO: 63 - DNA, 42 bp, Artificial Sequence
  Internal type primer for isothermal amplification mediated by SARS-Cov-2 E1 region loop
accacgaaagcaagaaaaagaagttcgtttcggaagagacag

SEQ ID NO: 64 - DNA, 44 bp, Artificial Sequence
  Internal type primer for isothermal amplification mediated by SARS-Cov-2 E1 region loop
ttgctagttacactagccatccttaggttttacaagactcacgt

SEQ ID NO: 65 - DNA, 18 bp, Artificial Sequence
  Loop type primer for isothermal amplification mediated by SARS-Cov-2 E1 region loop
cgctattaactattaacg

SEQ ID NO: 66 - DNA, 19 bp, Artificial Sequence
  Loop type primer for isothermal amplification mediated by SARS-Cov-2 E1 region loop
gcgcttcgattgtgtgcgt

SEQ ID NO: 67 - DNA, 18 bp, Artificial Sequence
  External type primer for isothermal mediated amplification by SARS-Cov-2 As1 region loop
cggtggacaaattgtcac

SEQ ID NO: 68 - DNA, 22 bp, Artificial Sequence
  External type primer for isothermal mediated amplification by SARS-Cov-2 As1 region loop
cttctctggatttaacacactt

SEQ ID NO: 69 - DNA, 51 bp, Artificial Sequence
  Internal type primer for isothermal amplification mediated by SARS-Cov-2 As1 region loop
tcagcacacaaagccaaaaatttatttttctgtgcaaaggaaattaaggag

SEQ ID NO: 70 - DNA, 49 bp, Artificial Sequence
  Internal type primer for isothermal amplification mediated by SARS-Cov-2 As1 region loop
tattggtggagctaaacttaaagccttttctgtacaatccctttgagtg

SEQ ID NO: 71 - DNA, 28 bp, Artificial Sequence
  Loop type primer for isothermal amplification mediated by SARS-Cov-2 As1 region loop
ttacaagcttaaagaatgtctgaacact

SEQ ID NO: 72 - DNA, 27 bp, Artificial Sequence
  Loop type primer for isothermal amplification mediated by SARS-Cov-2 As1 region loop
ttgaatttaggtgaaacatttgtcacg